European Patent Specification EP 3 684 936 B1, published December 6, 2023. Title: Method of production of barley plants producing antimicrobial peptides. Applicant: Univerzita Palackeho v Olomouci. The sequence listing filed with the application follows.

SEQUENCE LISTING (26 sequences)

SEQ ID NO: 1 - DNA, 180 bp, Artificial
  ZmCKX1sp_LL-37_KDEL
atggccgttgtttactacctcctcctcgccggcctcattgcctgctctcacgccctcctcggcgatttcttccgcaagtccaaggagaagatcggcaaggagttcaagaggatcgtccagaggatcaaggacttcctccgcaacctcgtgccaaggaccgagagcaaggacgagctttga

SEQ ID NO: 2 - DNA, 261 bp, Artificial
  ZmCKX1sp_(GGGGS)2_6xHis_ (GGGGS)2_LL-37
atggccgttgtttactacctcctcctcgccggcctcattgcctgctcccacgctggcggcggcggctccggcggcgggggcagccaccatcaccatcatcatggcgggggcggcagcggggggggcggctcagatgacgacgacaagctccttggcgacttcttccgcaagtccaaggagaagatcggcaaggagttcaagaggatcgtccagaggatcaaggacttcctgaggaacctcgtgccgaggaccgagtcttga

SEQ ID NO: 3 - DNA, 1359 bp, Artificial
  ZmCKX1sp_6xHis_MBP_LL-37_KDEL
atggccgtggtgtactacctcctcctcgccggcctgatcgcctgctcccacgcgcaccaccaccatcaccataagatcgaggagggcaagctcgtcatctggatcaacggcgacaagggctacaacggcctcgccgaggtgggcaagaagttcgagaaggacaccggcatcaaggtgaccgtcgagcacccagataagctggaggagaagttcccgcaggtcgccgccaccggcgacggcccggatatcatcttctgggcccacgacaggttcggcggctacgcccagtccggcctcctcgccgagatcaccccggacaaggccttccaggataagctctacccgttcacctgggacgccgtgaggtacaacggcaagctcattgcctacccgattgccgtcgaggccctctccctgatctacaacaaggacctcctcccgaacccgcccaagacctgggaggagatcccggccctcgacaaggagctgaaggccaagggcaagtccgccctcatgttcaacctccaggagccgtacttcacctggccactcattgcggccgacggggggtacgccttcaagtacgagaacggcaagtacgacatcaaggacgtgggcgtggacaacgctggcgccaaggcgggcctcaccttcctcgtggatctcatcaagaacaagcacatgaacgccgacaccgactactcgatcgccgaggccgccttcaacaagggcgagaccgccatgaccattaacggcccgtgggcctggtccaacatcgacacctctaaggtgaactacggcgtgaccgtgctcccgaccttcaagggccagccgtccaagccgttcgtgggcgtgctctccgccggcatcaacgccgcctccccgaacaaggagctggccaaggagttcctggagaactacctcctcaccgacgagggcctggaggccgtgaacaaggacaagccgctcggcgccgtggccctcaagtcctacgaggaggagctggcgaaggacccgaggatcgccgcgaccatggagaacgcccagaagggcgagatcatgccgaacatcccgcagatgtccgccttctggtacgccgtcaggaccgccgtgattaacgccgccagcggcaggcagaccgtggacgaggccctgaaggacgcccagaccaactcttcctcgaacaataacaataacaacaataataacaacctcggcgacgacgacgacaagctcctcggcgacttcttccgcaagtccaaggagaagatcggcaaggagttcaagaggatcgtccagaggatcaaggacttcctccgcaacctcgtgccaaggaccgagtccaaggatgagctgtga

SEQ ID NO: 4 - DNA, 207 bp, Artificial
  OsCht1sp_6xHis_LL-37
atgagggctctcgccgtggtggtggtcgccaccgccttcgctgtggtggccgtgaggggccaccatcaccatcatcatgacgacgacgataagctcctcggcgacttcttccgcaagtccaaggagaagatcggcaaggagttcaagaggatcgtccagaggatcaaggacttcctgaggaacctcgtgccgaggaccgagtcttga

SEQ ID NO: 5 - DNA, 57 bp, Artificial
  ZmCKX1sp
atggccgttgtttactacctcctcctcgccggcctcattgcctgctctcacgcctga

SEQ ID NO: 6 - DNA, 63 bp, Artificial
  OsCht1sp
atgagggctctcgccgtggtggtggtcgccaccgccttcgctgtggtggccgtgaggggctga

SEQ ID NO: 7 - DNA, 18 bp, Artificial
  KDEL
atgaaggatgagctgtga

SEQ ID NO: 8 - DNA, 1152 bp, Artificial
  MBP
atgaagatcgaggagggcaagctcgtcatctggatcaacggcgacaagggctacaacggcctcgccgaggtgggcaagaagttcgagaaggacaccggcatcaaggtgaccgtcgagcacccagataagctggaggagaagttcccgcaggtcgccgccaccggcgacggcccggatatcatcttctgggcccacgacaggttcggcggctacgcccagtccggcctcctcgccgagatcaccccggacaaggccttccaggataagctctacccgttcacctgggacgccgtgaggtacaacggcaagctcattgcctacccgattgccgtcgaggccctctccctgatctacaacaaggacctcctcccgaacccgcccaagacctgggaggagatcccggccctcgacaaggagctgaaggccaagggcaagtccgccctcatgttcaacctccaggagccgtacttcacctggccactcattgcggccgacggggggtacgccttcaagtacgagaacggcaagtacgacatcaaggacgtgggcgtggacaacgctggcgccaaggcgggcctcaccttcctcgtggatctcatcaagaacaagcacatgaacgccgacaccgactactcgatcgccgaggccgccttcaacaagggcgagaccgccatgaccattaacggcccgtgggcctggtccaacatcgacacctctaaggtgaactacggcgtgaccgtgctcccgaccttcaagggccagccgtccaagccgttcgtgggcgtgctctccgccggcatcaacgccgcctccccgaacaaggagctggccaaggagttcctggagaactacctcctcaccgacgagggcctggaggccgtgaacaaggacaagccgctcggcgccgtggccctcaagtcctacgaggaggagctggcgaaggacccgaggatcgccgcgaccatggagaacgcccagaagggcgagatcatgccgaacatcccgcagatgtccgccttctggtacgccgtcaggaccgccgtgattaacgccgccagcggcaggcagaccgtggacgaggccctgaaggacgcccagaccaactcttcctcgaacaataacaataacaacaataataacaacctcggctga

SEQ ID NO: 9 - DNA, 24 bp, Artificial
  6xHis
atgcaccatcaccatcatcattga

SEQ ID NO: 10 - DNA, 30 bp, Artificial
  8xHis
atgcaccatcaccatcatcatcatcattga

SEQ ID NO: 11 - DNA, 306 bp, Artificial
  SUMOstar
atgtcccttcaggactccgaggtgaaccaggaggccaagccagaggttaagcctgaggtgaagcccgagacccacatcaacctcaaggtgtccgacggctcctccgagatcttcttcaagatcaagaagaccaccccgctcaggcgcctcatggaggccttcgccaagaggcagggcaaggagatggattccctcaccttcctctacgacggcatcgagatccaggccgatcagaccccagaggacctcgacatggaggacaacgacatcattgaggcccaccgcgagcagattggcggcctttga

SEQ ID NO: 12 - DNA, 291 bp, Artificial
  HvSUMO
atgtctggcgttaccgccgacgaggataagaagccagccggcgacggcggcggcgctcatatcaacctcaaggttaagggccaggacggcaacgaggtgttcttcaggatcaagaggtccacccagctcaagaagctcatgaacgcctactgcgacaggcagtccgtggacctcaactcgatcgccttcctgttcgatggcaggcgcctcaggggcgagcagaccccagacgagcttgagatggaggagggcgacgagattgacgccatgcttcaccagaccggcggctga

SEQ ID NO: 13 - DNA, 303 bp, Artificial
  DAMP4
atggagccgtccatgaagcagctcgccgattccctccaccagctcgccaggcaggtttccaggcttgagcacgccgagcctagcatgaagcagcttgctgacagcctccatcagcttgcccgccaggtgtcacgccttgagcatgctgagccatcgatgaagcagctggcggactctctgcatcagctggctaggcaggtcagcaggcttgagcatgcggagccttccatgaagcagcttgcggatagccttcaccagctggcgcggcaggttagccgccttgagcacgcggatccatcttga

SEQ ID NO: 14 - DNA, 36 bp, Artificial
  (GGGGS)2
atgggcggcggcggctccggcggcgggggcagctga

SEQ ID NO: 15 - DNA, 1100 bp, Artificial
  B1 hordein promotor::ZmCKX1sp_LL-37_KDEL::Nos terminator
tttaaagtcgacgtgcaggtgtatgagtcattgttatgatctataggtgtcagtttatcttatcatctgggtgatcaatacaggcccaggttttataaaaaccagtcgagtcgagaagaaccgtccacatgtaaagctttaacaacccacacattgattgcaacttagtcctacacaagttttccattcttgtttcaggctaacaacctatacaaggttccaaaatcatgcaaaagtgatgctaggttgataatgtgtgacatgtaaagtgaataaggtgagtcatgcataccaaacctcgggatttctatactttgtgtatgatcatatgcacaactaaaaggcaactttgattatcaattgaaaagtaccgcttgtagcttgtgcaacctaacacaatgtccaaaaatccatttgcaaaagcatccaaacacaattgttaaagctgttcaaacaaacaaagaagagatgaagcctggctactataaataggcaggtagtatagagatctacacaagcacaagcatcaaaaccaagaaacactagttaacaccaatccactgtcgacggtaccggatccgccaccatggccgttgtttactacctcctcctcgccggcctcattgcctgctctcacgccctcctcggcgatttcttccgcaagtccaaggagaagatcggcaaggagttcaagaggatcgtccagaggatcaaggacttcctccgcaacctcgtgccaaggaccgagagcaaggacgagctttgactcgagccttggtctagagagctcagtcaagcaggatcgttcaaacatttggcaataaagtttcttaagattgaatcctgttgccggtcttgcgatgattatcatataatttctgttgaattacgttaagcatgtaataattaacatgtaatgcatgacgttatttatgagatgggtttttatgattagagtcccgcaattatacatttaatacgcgatagaaaacaaaatatagcgcgcaaactaggataaattatcgcgcgcggtgtcatctatgttactagatcgaccggcatgcaagctgatatgagctcgcatgcgcggccgcgatatc

SEQ ID NO: 16 - DNA, 2618 bp, Artificial
  ubiquitin promotor::ZmCKX1sp_LL-37_KDEL::Nos terminator
gtgcagcgtgacccggtcgtgcccctctctagagataatgagcattgcatgtctaagttataaaaaattaccacatattttttttgtcacacttgtttgaagtgcagtttatctatctttatacatatatttaaactttactctacgaataatataatctatagtactacaataatatcagtgttttagagaatcatataaatgaacagttagacatggtctaaaggacaattgagtattttgacaacaggactctacagttttatctttttagtgtgcatgtgttctcctttttttttgcaaatagcttcacctatataatacttcatccattttattagtacatccatttagggtttagggttaatggtttttatagactaatttttttagtacatctattttattctattttagcctctaaattaagaaaactaaaactctattttagtttttttatttaataatttagatataaaatagaataaaataaagtgactaaaaattaaacaaataccctttaagaaattaaaaaaactaaggaaacatttttcttgtttcgagtagataatgccagcctgttaaacgccgtcgacgagtctaacggacaccaaccagcgaaccagcagcgtcgcgtcgggccaagcgaagcagacggcacggcatctctgtcgctgcctctggacccctctcgagagttccgctccaccgttggacttgctccgctgtcggcatccagaaattgcgtgtcggacggcagacgtgagccggcacggcaggcggcctcctcctcctctcacggcaccggcagctacgggggattcctttcccaccgctccttcgctttcccttcctcgcccgccgtaataaatagacaccccctccacaccctctttccccaacctcgtgttgttcggagcgcacacacacacaaccagatctcccccaaatccacccgtcggcacctccgcttcaaggtacgccgctcgtcctccccccccccccctctctaccttctctagatcggcgttccggtccatggttagggcccggtagttctacttctgttcatgtttgtgttagatccgtgtttgtgttagatccgtgctgctagcgttcgtacacggatgcgacctgtacgtcagacacgttctgattgctaacttgccagtgtttctctttggggaatcctgggatggctctagccgttccgcagacgggatcgatttcatgatttttttttgtttcgttgcatagggtttggtttgcccttttcctttatttcaatatatgccgtgcacttgtttgtcgggtcatcttttcatgcttttttttgtcttggttgtgatgatgtggtctggttgggcggtcgttctagatcggagtagaattaattctgtttcaaactacctggtggatttattaattttggatctgtatgtgtgtgccatacatattcatagttacgaattgaagatgatggatggaaatatcgatctaggataggtatacatgttgatgcgggttttactgatgcatatacagagatgctttttgttcgcttggttgtgatgatgtggtgtggttgggcggtcgttcattcgttctagatcggagtagaatactgtttcaaactacctggtgtatttattaattttggaactgtatgtgtgtgtcatacatcttcatagttacgagtttaagatggatggaaatatcgatctaggataggtatacatgttgatgtgggttttactgatgcatatacatgatggcatatgcagcatctattcatatgctctaaccttgagtacctatctattataataaacaagtatgttttataattattttgatcttgatatacttggatgatggcatatgcagcagctatatgtggatttttttagccctgccttcatacgctatttatttgcttggtactgtttcttttgtcgatgctcaccctgttgtttggtgttacttcgcccatcacaagtttgtacaaaaaagcaggctggcgccggaaccaattcagtcgaccgtacgggatccgccaccatggccgttgtttactacctcctcctcgccggcctcattgcctgctctcacgccctcctcggcgatttcttccgcaagtccaaggagaagatcggcaaggagttcaagaggatcgtccagaggatcaaggacttcctccgcaacctcgtgccaaggaccgagagcaaggacgagctttgactcgaggaattcgcggccgcactcgagatatctagacccagctttcttgtacaaagtggtgatgggggatccactagttctagaattcgattgagtcaagcaggatcgttcaaacatttggcaataaagtttcttaagattgaatcctgttgccggtcttgcgatgattatcatataatttctgttgaattacgttaagcatgtaataattaacatgtaatgcatgacgttatttatgagatgggtttttatgattagagtcccgcaattatacatttaatacgcgatagaaaacaaaatatagcgcgcaaactaggataaattatcgcgcgcggtgtcatctatgttactagatcgaccggcatgcaagctgatat

SEQ ID NO: 17 - DNA, 1181 bp, Artificial
  B1 hordein promotor::ZmCKX1sp_(GGGGS)2_6xHis_(GGGGS)2_LL-37::Nos terminator
tttaaagtcgacgtgcaggtgtatgagtcattgttatgatctataggtgtcagtttatcttatcatctgggtgatcaatacaggcccaggttttataaaaaccagtcgagtcgagaagaaccgtccacatgtaaagctttaacaacccacacattgattgcaacttagtcctacacaagttttccattcttgtttcaggctaacaacctatacaaggttccaaaatcatgcaaaagtgatgctaggttgataatgtgtgacatgtaaagtgaataaggtgagtcatgcataccaaacctcgggatttctatactttgtgtatgatcatatgcacaactaaaaggcaactttgattatcaattgaaaagtaccgcttgtagcttgtgcaacctaacacaatgtccaaaaatccatttgcaaaagcatccaaacacaattgttaaagctgttcaaacaaacaaagaagagatgaagcctggctactataaataggcaggtagtatagagatctacacaagcacaagcatcaaaaccaagaaacactagttaacaccaatccactgtcgacggtaccggatccgccaccatggccgttgtttactacctcctcctcgccggcctcattgcctgctcccacgctggcggcggcggctccggcggcgggggcagccaccatcaccatcatcatggcgggggcggcagcggggggggcggctcagatgacgacgacaagctccttggcgacttcttccgcaagtccaaggagaagatcggcaaggagttcaagaggatcgtccagaggatcaaggacttcctgaggaacctcgtgccgaggaccgagtcttgactcgagccttggtctagagagctcagtcaagcaggatcgttcaaacatttggcaataaagtttcttaagattgaatcctgttgccggtcttgcgatgattatcatataatttctgttgaattacgttaagcatgtaataattaacatgtaatgcatgacgttatttatgagatgggtttttatgattagagtcccgcaattatacatttaatacgcgatagaaaacaaaatatagcgcgcaaactaggataaattatcgcgcgcggtgtcatctatgttactagatcgaccggcatgcaagctgatatgagctcgcatgcgcggccgcgatatc

SEQ ID NO: 18 - DNA, 2699 bp, Artificial
  ubiquitin promotor::ZmCKX1sp_(GGGGS)2_6xHis_ (GGGGS)2_LL-37::Nos terminator
gtgcagcgtgacccggtcgtgcccctctctagagataatgagcattgcatgtctaagttataaaaaattaccacatattttttttgtcacacttgtttgaagtgcagtttatctatctttatacatatatttaaactttactctacgaataatataatctatagtactacaataatatcagtgttttagagaatcatataaatgaacagttagacatggtctaaaggacaattgagtattttgacaacaggactctacagttttatctttttagtgtgcatgtgttctcctttttttttgcaaatagcttcacctatataatacttcatccattttattagtacatccatttagggtttagggttaatggtttttatagactaatttttttagtacatctattttattctattttagcctctaaattaagaaaactaaaactctattttagtttttttatttaataatttagatataaaatagaataaaataaagtgactaaaaattaaacaaataccctttaagaaattaaaaaaactaaggaaacatttttcttgtttcgagtagataatgccagcctgttaaacgccgtcgacgagtctaacggacaccaaccagcgaaccagcagcgtcgcgtcgggccaagcgaagcagacggcacggcatctctgtcgctgcctctggacccctctcgagagttccgctccaccgttggacttgctccgctgtcggcatccagaaattgcgtgtcggacggcagacgtgagccggcacggcaggcggcctcctcctcctctcacggcaccggcagctacgggggattcctttcccaccgctccttcgctttcccttcctcgcccgccgtaataaatagacaccccctccacaccctctttccccaacctcgtgttgttcggagcgcacacacacacaaccagatctcccccaaatccacccgtcggcacctccgcttcaaggtacgccgctcgtcctccccccccccccctctctaccttctctagatcggcgttccggtccatggttagggcccggtagttctacttctgttcatgtttgtgttagatccgtgtttgtgttagatccgtgctgctagcgttcgtacacggatgcgacctgtacgtcagacacgttctgattgctaacttgccagtgtttctctttggggaatcctgggatggctctagccgttccgcagacgggatcgatttcatgatttttttttgtttcgttgcatagggtttggtttgcccttttcctttatttcaatatatgccgtgcacttgtttgtcgggtcatcttttcatgcttttttttgtcttggttgtgatgatgtggtctggttgggcggtcgttctagatcggagtagaattaattctgtttcaaactacctggtggatttattaattttggatctgtatgtgtgtgccatacatattcatagttacgaattgaagatgatggatggaaatatcgatctaggataggtatacatgttgatgcgggttttactgatgcatatacagagatgctttttgttcgcttggttgtgatgatgtggtgtggttgggcggtcgttcattcgttctagatcggagtagaatactgtttcaaactacctggtgtatttattaattttggaactgtatgtgtgtgtcatacatcttcatagttacgagtttaagatggatggaaatatcgatctaggataggtatacatgttgatgtgggttttactgatgcatatacatgatggcatatgcagcatctattcatatgctctaaccttgagtacctatctattataataaacaagtatgttttataattattttgatcttgatatacttggatgatggcatatgcagcagctatatgtggatttttttagccctgccttcatacgctatttatttgcttggtactgtttcttttgtcgatgctcaccctgttgtttggtgttacttcgcccatcacaagtttgtacaaaaaagcaggctggcgccggaaccaattcagtcgaccgtacgggatccgccaccatggccgttgtttactacctcctcctcgccggcctcattgcctgctcccacgctggcggcggcggctccggcggcgggggcagccaccatcaccatcatcatggcgggggcggcagcggggggggcggctcagatgacgacgacaagctccttggcgacttcttccgcaagtccaaggagaagatcggcaaggagttcaagaggatcgtccagaggatcaaggacttcctgaggaacctcgtgccgaggaccgagtcttgactcgaggaattcgcggccgcactcgagatatctagacccagctttcttgtacaaagtggtgatgggggatccactagttctagaattcgattgagtcaagcaggatcgttcaaacatttggcaataaagtttcttaagattgaatcctgttgccggtcttgcgatgattatcatataatttctgttgaattacgttaagcatgtaataattaacatgtaatgcatgacgttatttatgagatgggtttttatgattagagtcccgcaattatacatttaatacgcgatagaaaacaaaatatagcgcgcaaactaggataaattatcgcgcgcggtgtcatctatgttactagatcgaccggcatgcaagctgatat

SEQ ID NO: 19 - DNA, 2282 bp, Artificial
  B1 hordein promotor::ZmCKX1sp_6xHis_MBP_LL-37_KDEL::Nos terminator
tttaaagtcgacgtgcaggtgtatgagtcattgttatgatctataggtgtcagtttatcttatcatctgggtgatcaatacaggcccaggttttataaaaaccagtcgagtcgagaagaaccgtccacatgtaaagctttaacaacccacacattgattgcaacttagtcctacacaagttttccattcttgtttcaggctaacaacctatacaaggttccaaaatcatgcaaaagtgatgctaggttgataatgtgtgacatgtaaagtgaataaggtgagtcatgcataccaaacctcgggatttctatactttgtgtatgatcatatgcacaactaaaaggcaactttgattatcaattgaaaagtaccgcttgtagcttgtgcaacctaacacaatgtccaaaaatccatttgcaaaagcatccaaacacaattgttaaagctgttcaaacaaacaaagaagagatgaagcctggctactataaataggcaggtagtatagagatctacacaagcacaagcatcaaaaccaagaaacactagttaacaccaatccactgtcgacggtaccggatccgcggcagcgatggccgtggtgtactacctcctcctcgccggcctgatcgcctgctcccacgcgcaccaccaccatcaccataagatcgaggagggcaagctcgtcatctggatcaacggcgacaagggctacaacggcctcgccgaggtgggcaagaagttcgagaaggacaccggcatcaaggtgaccgtcgagcacccagataagctggaggagaagttcccgcaggtcgccgccaccggcgacggcccggatatcatcttctgggcccacgacaggttcggcggctacgcccagtccggcctcctcgccgagatcaccccggacaaggccttccaggataagctctacccgttcacctgggacgccgtgaggtacaacggcaagctcattgcctacccgattgccgtcgaggccctctccctgatctacaacaaggacctcctcccgaacccgcccaagacctgggaggagatcccggccctcgacaaggagctgaaggccaagggcaagtccgccctcatgttcaacctccaggagccgtacttcacctggccactcattgcggccgacggggggtacgccttcaagtacgagaacggcaagtacgacatcaaggacgtgggcgtggacaacgctggcgccaaggcgggcctcaccttcctcgtggatctcatcaagaacaagcacatgaacgccgacaccgactactcgatcgccgaggccgccttcaacaagggcgagaccgccatgaccattaacggcccgtgggcctggtccaacatcgacacctctaaggtgaactacggcgtgaccgtgctcccgaccttcaagggccagccgtccaagccgttcgtgggcgtgctctccgccggcatcaacgccgcctccccgaacaaggagctggccaaggagttcctggagaactacctcctcaccgacgagggcctggaggccgtgaacaaggacaagccgctcggcgccgtggccctcaagtcctacgaggaggagctggcgaaggacccgaggatcgccgcgaccatggagaacgcccagaagggcgagatcatgccgaacatcccgcagatgtccgccttctggtacgccgtcaggaccgccgtgattaacgccgccagcggcaggcagaccgtggacgaggccctgaaggacgcccagaccaactcttcctcgaacaataacaataacaacaataataacaacctcggcgacgacgacgacaagctcctcggcgacttcttccgcaagtccaaggagaagatcggcaaggagttcaagaggatcgtccagaggatcaaggacttcctccgcaacctcgtgccaaggaccgagtccaaggatgagctgtgactcgagccttggtctagagagctcagtcaagcaggatcgttcaaacatttggcaataaagtttcttaagattgaatcctgttgccggtcttgcgatgattatcatataatttctgttgaattacgttaagcatgtaataattaacatgtaatgcatgacgttatttatgagatgggtttttatgattagagtcccgcaattatacatttaatacgcgatagaaaacaaaatatagcgcgcaaactaggataaattatcgcgcgcggtgtcatctatgttactagatcgaccggcatgcaagctgatatgagctcgcatgcgcggccgcgatatc

SEQ ID NO: 20 - DNA, 3800 bp, Artificial
  ubiquitin promotor::ZmCKX1sp_6xHis_MBP_LL-37_KDEL::Nos terminator
gtgcagcgtgacccggtcgtgcccctctctagagataatgagcattgcatgtctaagttataaaaaattaccacatattttttttgtcacacttgtttgaagtgcagtttatctatctttatacatatatttaaactttactctacgaataatataatctatagtactacaataatatcagtgttttagagaatcatataaatgaacagttagacatggtctaaaggacaattgagtattttgacaacaggactctacagttttatctttttagtgtgcatgtgttctcctttttttttgcaaatagcttcacctatataatacttcatccattttattagtacatccatttagggtttagggttaatggtttttatagactaatttttttagtacatctattttattctattttagcctctaaattaagaaaactaaaactctattttagtttttttatttaataatttagatataaaatagaataaaataaagtgactaaaaattaaacaaataccctttaagaaattaaaaaaactaaggaaacatttttcttgtttcgagtagataatgccagcctgttaaacgccgtcgacgagtctaacggacaccaaccagcgaaccagcagcgtcgcgtcgggccaagcgaagcagacggcacggcatctctgtcgctgcctctggacccctctcgagagttccgctccaccgttggacttgctccgctgtcggcatccagaaattgcgtgtcggacggcagacgtgagccggcacggcaggcggcctcctcctcctctcacggcaccggcagctacgggggattcctttcccaccgctccttcgctttcccttcctcgcccgccgtaataaatagacaccccctccacaccctctttccccaacctcgtgttgttcggagcgcacacacacacaaccagatctcccccaaatccacccgtcggcacctccgcttcaaggtacgccgctcgtcctccccccccccccctctctaccttctctagatcggcgttccggtccatggttagggcccggtagttctacttctgttcatgtttgtgttagatccgtgtttgtgttagatccgtgctgctagcgttcgtacacggatgcgacctgtacgtcagacacgttctgattgctaacttgccagtgtttctctttggggaatcctgggatggctctagccgttccgcagacgggatcgatttcatgatttttttttgtttcgttgcatagggtttggtttgcccttttcctttatttcaatatatgccgtgcacttgtttgtcgggtcatcttttcatgcttttttttgtcttggttgtgatgatgtggtctggttgggcggtcgttctagatcggagtagaattaattctgtttcaaactacctggtggatttattaattttggatctgtatgtgtgtgccatacatattcatagttacgaattgaagatgatggatggaaatatcgatctaggataggtatacatgttgatgcgggttttactgatgcatatacagagatgctttttgttcgcttggttgtgatgatgtggtgtggttgggcggtcgttcattcgttctagatcggagtagaatactgtttcaaactacctggtgtatttattaattttggaactgtatgtgtgtgtcatacatcttcatagttacgagtttaagatggatggaaatatcgatctaggataggtatacatgttgatgtgggttttactgatgcatatacatgatggcatatgcagcatctattcatatgctctaaccttgagtacctatctattataataaacaagtatgttttataattattttgatcttgatatacttggatgatggcatatgcagcagctatatgtggatttttttagccctgccttcatacgctatttatttgcttggtactgtttcttttgtcgatgctcaccctgttgtttggtgttacttcgcccatcacaagtttgtacaaaaaagcaggctggcgccggaaccaattcagtcgaccgtacgggatccgcggcagcgatggccgtggtgtactacctcctcctcgccggcctgatcgcctgctcccacgcgcaccaccaccatcaccataagatcgaggagggcaagctcgtcatctggatcaacggcgacaagggctacaacggcctcgccgaggtgggcaagaagttcgagaaggacaccggcatcaaggtgaccgtcgagcacccagataagctggaggagaagttcccgcaggtcgccgccaccggcgacggcccggatatcatcttctgggcccacgacaggttcggcggctacgcccagtccggcctcctcgccgagatcaccccggacaaggccttccaggataagctctacccgttcacctgggacgccgtgaggtacaacggcaagctcattgcctacccgattgccgtcgaggccctctccctgatctacaacaaggacctcctcccgaacccgcccaagacctgggaggagatcccggccctcgacaaggagctgaaggccaagggcaagtccgccctcatgttcaacctccaggagccgtacttcacctggccactcattgcggccgacggggggtacgccttcaagtacgagaacggcaagtacgacatcaaggacgtgggcgtggacaacgctggcgccaaggcgggcctcaccttcctcgtggatctcatcaagaacaagcacatgaacgccgacaccgactactcgatcgccgaggccgccttcaacaagggcgagaccgccatgaccattaacggcccgtgggcctggtccaacatcgacacctctaaggtgaactacggcgtgaccgtgctcccgaccttcaagggccagccgtccaagccgttcgtgggcgtgctctccgccggcatcaacgccgcctccccgaacaaggagctggccaaggagttcctggagaactacctcctcaccgacgagggcctggaggccgtgaacaaggacaagccgctcggcgccgtggccctcaagtcctacgaggaggagctggcgaaggacccgaggatcgccgcgaccatggagaacgcccagaagggcgagatcatgccgaacatcccgcagatgtccgccttctggtacgccgtcaggaccgccgtgattaacgccgccagcggcaggcagaccgtggacgaggccctgaaggacgcccagaccaactcttcctcgaacaataacaataacaacaataataacaacctcggcgacgacgacgacaagctcctcggcgacttcttccgcaagtccaaggagaagatcggcaaggagttcaagaggatcgtccagaggatcaaggacttcctccgcaacctcgtgccaaggaccgagtccaaggatgagctgtgactcgaggaattcgcggccgcactcgagatatctagacccagctttcttgtacaaagtggtgatgggggatccactagttctagaattcgattgagtcaagcaggatcgttcaaacatttggcaataaagtttcttaagattgaatcctgttgccggtcttgcgatgattatcatataatttctgttgaattacgttaagcatgtaataattaacatgtaatgcatgacgttatttatgagatgggtttttatgattagagtcccgcaattatacatttaatacgcgatagaaaacaaaatatagcgcgcaaactaggataaattatcgcgcgcggtgtcatctatgttactagatcgaccggcatgcaagctgatat

SEQ ID NO: 21 - DNA, 1127 bp, Artificial
  B1 hordein promotor::OsCht1sp_6xHis_LL-37::Nos terminator
tttaaagtcgacgtgcaggtgtatgagtcattgttatgatctataggtgtcagtttatcttatcatctgggtgatcaatacaggcccaggttttataaaaaccagtcgagtcgagaagaaccgtccacatgtaaagctttaacaacccacacattgattgcaacttagtcctacacaagttttccattcttgtttcaggctaacaacctatacaaggttccaaaatcatgcaaaagtgatgctaggttgataatgtgtgacatgtaaagtgaataaggtgagtcatgcataccaaacctcgggatttctatactttgtgtatgatcatatgcacaactaaaaggcaactttgattatcaattgaaaagtaccgcttgtagcttgtgcaacctaacacaatgtccaaaaatccatttgcaaaagcatccaaacacaattgttaaagctgttcaaacaaacaaagaagagatgaagcctggctactataaataggcaggtagtatagagatctacacaagcacaagcatcaaaaccaagaaacactagttaacaccaatccactgtcgacggtaccggatccgccaccatgagggctctcgccgtggtggtggtcgccaccgccttcgctgtggtggccgtgaggggccaccatcaccatcatcatgacgacgacgataagctcctcggcgacttcttccgcaagtccaaggagaagatcggcaaggagttcaagaggatcgtccagaggatcaaggacttcctgaggaacctcgtgccgaggaccgagtcttgactcgagccttggtctagagagctcagtcaagcaggatcgttcaaacatttggcaataaagtttcttaagattgaatcctgttgccggtcttgcgatgattatcatataatttctgttgaattacgttaagcatgtaataattaacatgtaatgcatgacgttatttatgagatgggtttttatgattagagtcccgcaattatacatttaatacgcgatagaaaacaaaatatagcgcgcaaactaggataaattatcgcgcgcggtgtcatctatgttactagatcgaccggcatgcaagctgatatgagctcgcatgcgcggccgcgatatc

SEQ ID NO: 22 - DNA, 1418 bp, Artificial
  AsGLO1p::8xHis_HBD2_KDEL::Nos terminator
tggaaagtcattttgcctcctgaactccagtgtttcctgtttattaaaaaaactaaaaactatacttataagtttgaaaagatcatgaaacaaaattgtaaaaattgctaatgatatatcccacaaacgtgcaaaatctcaattcgaagtgctttgtatttcgaactacacaaaaatgacaaagtgtgactttttatgtgattcgaaatcactatactacagatctacaattttgtcatttttgtgaagctaaaaatacacattatttcgaattgagatttttcatgtttgtgctatgaatcacaggctacatcctgatttatttttagaattttttggaacccaaaatatgttctagattattttttaaaaagtgggatcacttatgcccatacacacgaaatctccactcaattcttttatacattatctttctatatctactaacgtggattatacatcatagtaagtttcttactacatgtgctttcttgtgacaatgtggacacgactcttccacttttgggctttatgttgtattgatatactcatgacatggaattttgtccacacacgtagatccatccatatatattgttgtgcatagaacgaaacacaagcaagccattaaaaaggagtcacaagtgccacaaactgttgtaggaagtacaactagtatgaggccttttatttgacgtcggacaatggccaagagctacatacaaaagatggtgctagatttgtgagtaagcaccagttgtaggcagaaaacaacacatatcttttgaggcaaagttatatctattcacatttaaaaccatgatctgttgagtcaccatgaatatctttttatctatgttaataattacatgtcatcatgtttatcctggactactttttatggctataaaatcaaacttacaattaggaaactagcaccaatccaccttctacaatctcggatccgtcctaaagccgtacggaattcgccaccatgcaccaccatcatcatcaccatcacgacgacgatgacaaggacccggtgacctgcctcaagtctggcgccatttgccacccagtgttctgcccaaggcgctacaagcagatcggcacgtgcggcctcccaggcaccaagtgctgcaagaagccaaactgactcgagcctaggtcaaacatttggcaataaagtttcttaagattgaatcctgttgccggtcttgcgatgattatcatataatttctgttgaattacgttaagcatgtaataattaacatgtaatgcatgacgttatttatgagatgggtttttatgattagagtcccgcaattatacatttaatacgcgatagaaaacaaaatatagcgcgcaaactaggataaattatcgcgcgcggtgtcatctatgttactagatcggg

SEQ ID NO: 23 - DNA, 2757 bp, Artificial
  TIp::PEX_KDEL::Nos terminator
gtcgacgcatgtgtcatctcattctgaaacgtgtggtgctgagacggttggaaatatgccctagaggtaatgataaatagttattattatatttcttgtttcaagataatcatttattattcatgctataattatattgaatgaaaacatagatacatgtgtgaatacattgacgaaacaatgtccttagcaagcctctagttggctagccagttgatcaaggatagtcaaggttttctgactatgtgcaagtgttgtcacttgataactggatcacatcattaggagaatcatgtgatggactagacccaaactatgaatgtagcatattgatcgtgtcattttgttgctattgttttctgcgtgtcaagtatttattcctatgaccatgagatcatataactcactggtaccggaggaataccttgtgtgtatcaaacgtcgcaacgtaactgagtgactataaaggtgctctacaggtatctctgaaggtgtccgttgagttagtatggatcaagactaggatttgccactccgtgtgacgtagaggtatctcggcccactcggtaatacaacatcacacacaagccttgcaagcaatgtgactaagtttaagtcacgggatcttgtattaccgaacgagaaaagagacatggatgctagtagatttctttttgtagagcacctcacaactagacgggccctgaaacacctatacttatatttagtatacaaaatgtttgtcctgaaacaatacgtgagttgcagaaaacgaagcgacttcgatagacgcaggaacacacgatggaacgaccacggagccgaaggacggccgcgcgatcggtcggtactagataatattttcccaaaagataatgcatggatgctagtagacttattttcagaagtactatacatacgatacgatacgacatatcataccaaaatcgtatgccaaattatcgtatatagagtaattccgtttcttttttgtcccggtggatctgaaataaccactttctggaaaatcttggaaatttaggttttttctgcccgaatgaatttaaaggaactttgaatttgatttttttgctgtgtgaaaatatatataaagacgctaacctactgactaacgtaactccctcatgctcgactgatcggttgggtacactctttcgcccgccaggtcatgagattggatcctctcgatcggttgcagacatgatctcgactcataaaccaaacgagagtttacttgaagtgctagattacactacaaataaacatggaagagaatgacatgcagatgaactagggataattctgttatctcttttcgtagggttcttcttgaacctcgactggcagcatgggatgaagtactcactcgtttggaggctcgttcagctgtcacatggatgctagtagatttcttttcgtagagcccctcacaaccagacgggccccgaaacacctatacttatatccagtataaaaaatgtctgtcctgaaacaatacgtgagttgcaggaaaacgaaagcggcttcgatagacgcaggaacacacgaacgaacggccgcgcgattggtcggtactagataatattttcccaaaagataatgcatggatgctactagatttttttcagaagtactctgcatacgatacgatatgacatatcatacaaaatcgtatgccaaattatcgtatttagagttaattatgtttcttttttgttcgagggatctgaaataaccggtttctggaaaatcttgtaaattcaaggtttttccgcccgaatgaatttaaacaaactttgaatttgatttttttgcagtgtgaaaatatatataaagatgctaacctactgactaacgtaactccctcatgctcgactgatcggttgcgtagaccctgtcgcccgccaggtcatgagattggatcctctcggctgcagacatgatctccactcataaagcaaacgagagtttacttgaagtgttagattacacatttacactacgaataaacatggaagagaatggcatgcagatgaaccagggatgtagcgtagtatgataagataactcatgccaagcacactgagaaaggtaggaaccgaggaaatatggttattcttctactcaaaccccaacttttgcattcccctccgaatattgttagcacaaagctccaaattctgtcagcaaaaaaggttatcaaagctaccctttaatcaaaatttccatgcagcggcactccaacaactaacagaaagtcagaaagcacttcggtacttacgatgccagctgcttgtcacttcacatttcactatatatatacatgtgatacgcctcgcttgctccaacaacatcccttcaatttgataacacgtacggaattcgccaccatgggcatcggcaagttcctcaagaaggccaagaagttcggcaaggccttcgtgaagatcctgaagaagaaggacgagctttgactcgagcctaggtcaaacatttggcaataaagtttcttaagattgaatcctgttgccggtcttgcgatgattatcatataatttctgttgaattacgttaagcatgtaataattaacatgtaatgcatgacgttatttatgagatgggtttttatgattagagtcccgcaattatacatttaatacgcgatagaaaacaaaatatagcgcgcaaactaggataaattatcgcgcgcggtgtcatctatgttactagatcggg

SEQ ID NO: 24 - protein, 41 aa, Artificial
  chimeric LL-37
LLGDFFRKSKEKIGKEFKRIVQRIKDFLRNLVPRTESKDEL

SEQ ID NO: 25 - protein, 48 aa, Artificial
  chimeric LL-37
HHHHHHDDDDKLLGDFFRKSKEKIGKEFKRIVQRIKDFLRNLVPRTES

SEQ ID NO: 26 - protein, 68 aa, Artificial
  chimeric LL-37
GGGGSGGGGSHHHHHHGGGGSGGGGSDDDDKLLGDFFRKSKEKIGKEFKRIVQRIKDFLRNLVPRTES